European Patent Specification EP 3 582 754 B1, published January 10, 2024. Title: COMPOSITION AND METHODS FOR PREVENTING RADIATION INJURY AND PROMOTING TISSUE REGENERATION. Applicant: FirstString Research, Inc. Ghatnekar, Gautam. The sequence listing filed with the application follows.

SEQUENCE LISTING (91 sequences)

SEQ ID NO: 1 - protein, 20 aa, Artificial Sequence
  Description of Artificial Sequences; note = synthetic construct
PSSRASSRASSRPRPDDLEI

SEQ ID NO: 2 - protein, 9 aa, Artificial Sequence
  Description of Artificial Sequences; note = synthetic construct
RPRPDDLEI

SEQ ID NO: 3 - protein, 9 aa, Artificial Sequence
  Description of Artificial Sequences; note = synthetic construct
RPRPDDLEV

SEQ ID NO: 4 - protein, 9 aa, Artificial Sequence
  Description of Artificial Sequences; note = synthetic construct
RPRPDDVPV

SEQ ID NO: 5 - protein, 9 aa, Artificial Sequence
  Description of Artificial Sequences; note = synthetic construct
KARSDDLSV

SEQ ID NO: 6 - DNA, 27 bp, Artificial Sequence
  Description of Artificial Sequences; note = synthetic construct
agacctcggcctgatgacctggagatt

SEQ ID NO: 7 - protein, 16 aa, Artificial Sequence
  Description of Artificial Sequences; note = synthetic construct
RQPKIWFPNRRKPWKK

SEQ ID NO: 8 - protein, 36 aa, Artificial Sequence
  Description of Artificial Sequences; note = synthetic construct
RQPKIWFPNRRKPWKKPSSRASSRASSRPRPDDLEI

SEQ ID NO: 9 - protein, 25 aa, Artificial Sequence
  Description of Artificial Sequences; note = synthetic construct
RQPKIWFPNRRKPWKKRPRPDDLEI

SEQ ID NO: 10 - protein, 25 aa, Artificial Sequence
  Description of Artificial Sequences; note = synthetic construct
RQPKIWFPNRRKPWKKRPRPDDLEV

SEQ ID NO: 11 - protein, 25 aa, Artificial Sequence
  Description of Artificial Sequences; note = synthetic construct
RQPKIWFPNRRKPWKKRPRPDDVPV

SEQ ID NO: 12 - protein, 25 aa, Artificial Sequence
  Description of Artificial Sequences; note = synthetic construct
RQPKIWFPNRRKPWKKKARSDDLSV

SEQ ID NO: 13 - DNA, 74 bp, Artificial Sequence
  Description of Artificial Sequences; note = synthetic construct
cggcagcccaagatctggttccccaaccggcggaagccctggaagaagcggcccggcccgacgacctggagatc

SEQ ID NO: 14 - protein, 11 aa, Artificial Sequence
  Description of Artificial Sequences; note = synthetic construct
GRKKRRQRPPQ

SEQ ID NO: 15 - protein, 16 aa, Artificial Sequence
  Description of Artificial Sequences; note = synthetic construct
RQIKIWFQNRRMKWKK

SEQ ID NO: 16 - protein, 16 aa, Artificial Sequence
  Description of Artificial Sequences; note = synthetic construct
RQIAIWFQNRRMKWAA

SEQ ID NO: 17 - protein, 9 aa, Artificial Sequence
  Description of Artificial Sequences; note = synthetic construct
RKKRRQRRR

SEQ ID NO: 18 - protein, 21 aa, Artificial Sequence
  Description of Artificial Sequences; note = synthetic construct
TRSSRAGLQFPVGRVHRLLRK

SEQ ID NO: 19 - protein, 26 aa, Artificial Sequence
  Description of Artificial Sequences; note = synthetic construct
GWTLNSAGYLLGKINKALAALAKKIL

SEQ ID NO: 20 - protein, 18 aa, Artificial Sequence
  Description of Artificial Sequences; note = synthetic construct
KLALKLALKALKAALKLA

SEQ ID NO: 21 - protein, 16 aa, Artificial Sequence
  Description of Artificial Sequences; note = synthetic construct
AAVALLPAVLLALLAP

SEQ ID NO: 22 - protein, 10 aa, Artificial Sequence
  Description of Artificial Sequences; note = synthetic construct
VPMLKPMLKE

SEQ ID NO: 23 - protein, 28 aa, Artificial Sequence
  Description of Artificial Sequences; note = synthetic construct
MANLGYWLLALFVTMWTDVGLCKKRPKP

SEQ ID NO: 24 - protein, 18 aa, Artificial Sequence
  Description of Artificial Sequences; note = synthetic construct
LLIILRRRIRKQAHAHSK

SEQ ID NO: 25 - protein, 21 aa, Artificial Sequence
  Description of Artificial Sequences; note = synthetic construct
KETWWETWWTEWSQPKKKRKV

SEQ ID NO: 26 - protein, 18 aa, Artificial Sequence
  Description of Artificial Sequences; note = synthetic construct
RGGRLSYSRRRFSTSTGR

SEQ ID NO: 27 - protein, 15 aa, Artificial Sequence
  Description of Artificial Sequences; note = synthetic construct
SDLWEMMMVSLACQY

SEQ ID NO: 28 - protein, 12 aa, Artificial Sequence
  Description of Artificial Sequences; note = synthetic construct
TSPLNIHNGQKL

SEQ ID NO: 29 - protein, 19 aa, Artificial Sequence
  Description of Artificial Sequences; note = synthetic construct
PSRASSRASSRPRPDDLEI

SEQ ID NO: 30 - protein, 20 aa, Artificial Sequence
  Description of Artificial Sequences; note = synthetic construct
GSNKSTASSKSPDPKNSVWI

SEQ ID NO: 31 - protein, 20 aa, Artificial Sequence
  Description of Artificial Sequences; note = synthetic construct
GSNKSSASSKSGDGKNSVWI

SEQ ID NO: 32 - protein, 21 aa, Artificial Sequence
  Description of Artificial Sequences; note = synthetic construct
GRASKASRASSGRARPEDLAI

SEQ ID NO: 33 - protein, 13 aa, Artificial Sequence
  Description of Artificial Sequences; note = synthetic construct
GSASSRDGKTVWI

SEQ ID NO: 34 - protein, 19 aa, Artificial Sequence
  Description of Artificial Sequences; note = synthetic construct
PRVSVPNFGRTQSSDSAYV

SEQ ID NO: 35 - protein, 19 aa, Artificial Sequence
  Description of Artificial Sequences; note = synthetic construct
PRMSMPNFGRTQSSDSAYV

SEQ ID NO: 36 - protein, 21 aa, Artificial Sequence
  Description of Artificial Sequences; note = synthetic construct
PRAGSEKGSASSRDGKTTVWI

SEQ ID NO: 37 - protein, 23 aa, Artificial Sequence
  Description of Artificial Sequences; note = synthetic construct
GYHSDKRRLSKASSKARSDDLSV

SEQ ID NO: 38 - protein, 19 aa, Artificial Sequence
  Description of Artificial Sequences; note = synthetic construct
PLSRLSKASSRARSDDLTV

SEQ ID NO: 39 - protein, 22 aa, Artificial Sequence
  Description of Artificial Sequences; note = synthetic construct
PNHVVSLTNNLIGRRVPTDLQI

SEQ ID NO: 40 - protein, 29 aa, Artificial Sequence
  Description of Artificial Sequences; note = synthetic construct
PSCVSSSAVLTTICSSDQVVPVGLSSFYM

SEQ ID NO: 41 - protein, 21 aa, Artificial Sequence
  Description of Artificial Sequences; note = synthetic construct
GRSSKASKSSGGRARAADLAI

SEQ ID NO: 42 - protein, 17 aa, Artificial Sequence
  Description of Artificial Sequences; note = synthetic construct
LCYLLIRYCSGKSKKPV

SEQ ID NO: 43 - protein, 18 aa, Artificial Sequence
  Description of Artificial Sequences; note = synthetic construct
GQKPPSRPSSSASKKQYV

SEQ ID NO: 44 - protein, 19 aa, Artificial Sequence
  Description of Artificial Sequences; note = synthetic construct
SSRASSRASSRPRPDDLEV

SEQ ID NO: 45 - protein, 9 aa, Artificial Sequence
  Description of Artificial Sequences; note = synthetic construct
RPKPDDLEI

SEQ ID NO: 46 - protein, 19 aa, Artificial Sequence
  Description of Artificial Sequences; note = synthetic construct
SSRASSRASSRPKPDDLEI

SEQ ID NO: 47 - protein, 9 aa, Artificial Sequence
  Description of Artificial Sequences; note = synthetic construct
RPKPDDLDI

SEQ ID NO: 48 - protein, 19 aa, Artificial Sequence
  Description of Artificial Sequences; note = synthetic construct
SSRASSRASSRPRPDDLDI

SEQ ID NO: 49 - protein, 19 aa, Artificial Sequence
  Description of Artificial Sequences; note = synthetic construct
SSRASTRASSRPRPDDLEI

SEQ ID NO: 50 - protein, 9 aa, Artificial Sequence
  Description of Artificial Sequences; note = synthetic construct
RPRPEDLEI

SEQ ID NO: 51 - protein, 19 aa, Artificial Sequence
  Description of Artificial Sequences; note = synthetic construct
SSRASSRASSRPRPEDLEI

SEQ ID NO: 52 - protein, 9 aa, Artificial Sequence
  Description of Artificial Sequences; note = synthetic construct
GDGKNSVWV

SEQ ID NO: 53 - protein, 23 aa, Artificial Sequence
  Description of Artificial Sequences; note = synthetic construct
SKAGSNKSTASSKSGDGKNSVWV

SEQ ID NO: 54 - protein, 18 aa, Artificial Sequence
  Description of Artificial Sequences; note = synthetic construct
GQKPPSRPSSSASKKLYV

SEQ ID NO: 55 - protein, 24 aa, Artificial Sequence
  Description of Artificial Sequences; note = synthetic construct
RQPKIWFPNRRKPWKIELDDPRPR

SEQ ID NO: 56 - protein, 20 aa, Artificial Sequence
  Description of Artificial Sequences; note = synthetic construct
GRKKRRQRPPQRPRPDDLEI

SEQ ID NO: 57 - protein, 25 aa, Artificial Sequence
  Description of Artificial Sequences; note = synthetic construct
RQIKIWFQNRRMKWKKRPRPDDLEI

SEQ ID NO: 58 - protein, 25 aa, Artificial Sequence
  Description of Artificial Sequences; note = synthetic construct
RQIAIWFQNRRMKWAARPRPDDLEI

SEQ ID NO: 59 - protein, 18 aa, Artificial Sequence
  Description of Artificial Sequences; note = synthetic construct
RKKRRQRRRRPRPDDLEI

SEQ ID NO: 60 - protein, 30 aa, Artificial Sequence
  Description of Artificial Sequences; note = synthetic construct
TRSSRAGLQFPVGRVHRLLRKRPRPDDLEI

SEQ ID NO: 61 - protein, 35 aa, Artificial Sequence
  Description of Artificial Sequences; note = synthetic construct
GWTLNSAGYLLGKINKALAALAKKILRPRPDDLEI

SEQ ID NO: 62 - protein, 27 aa, Artificial Sequence
  Description of Artificial Sequences; note = synthetic construct
KLALKLALKALKAALKLARPRPDDLEI

SEQ ID NO: 63 - protein, 25 aa, Artificial Sequence
  Description of Artificial Sequences; note = synthetic construct
AAVALLPAVLLALLAPRPRPDDLEI

SEQ ID NO: 64 - protein, 19 aa, Artificial Sequence
  Description of Artificial Sequences; note = synthetic construct
VPMLKPMLKERPRPDDLEI

SEQ ID NO: 65 - protein, 37 aa, Artificial Sequence
  Description of Artificial Sequences; note = synthetic construct
MANLGYWLLALFVTMWTDVGLCKKRPKPRPRPDDLEI

SEQ ID NO: 66 - protein, 27 aa, Artificial Sequence
  Description of Artificial Sequences; note = synthetic construct
LLIILRRRIRKQAHAHSKRPRPDDLEI

SEQ ID NO: 67 - protein, 30 aa, Artificial Sequence
  Description of Artificial Sequences; note = synthetic construct
KETWWETWWTEWSQPKKKRKVRPRPDDLEI

SEQ ID NO: 68 - protein, 27 aa, Artificial Sequence
  Description of Artificial Sequences; note = synthetic construct
RGGRLSYSRRRFSTSTGRRPRPDDLEI

SEQ ID NO: 69 - protein, 24 aa, Artificial Sequence
  Description of Artificial Sequences; note = synthetic construct
SDLWEMMMVSLACQYRPRPDDLEI

SEQ ID NO: 70 - protein, 21 aa, Artificial Sequence
  Description of Artificial Sequences; note = synthetic construct
TSPLNIHNGQKLRPRPDDLEI

SEQ ID NO: 71 - protein, 120 aa, Artificial Sequence
  Description of Artificial Sequences; note = synthetic construct
KGKSDPYHATSGALSPAKDCGSQKYAYFNGCSSPTAPLSPMSPPGYKLVTGDRNNSSCRNYNKQASEQNWANYSAEQNRMGQAGSTISNSHAQPFDFPDDNQNSKKLAAGHELQPLAIVD

SEQ ID NO: 72 - protein, 120 aa, Artificial Sequence
  Description of Artificial Sequences; note = synthetic construct
KTDPYSHSGTMSPSKDCGSPKYAYYNGCSSPTAPLSPMSPPGYKLVTGDRNNSSCRNYNKQASEQNWANYSAEQNRMGQAGSTISNSHAQPFDFADEHQNTKKLASGHELQPLTIVDQRP

SEQ ID NO: 73 - protein, 120 aa, Artificial Sequence
  Description of Artificial Sequences; note = synthetic construct
LGFGTIRDSLNSKRRELEDPGAYNYPFTWNTPSAPPGYNIAVKPDQIQYTELSNAKIAYKQNKANTAQEQQYGSHEENLPADLEALQREIRMAQERLDLAVQAYSHQNNPHGPREKKAKV

SEQ ID NO: 74 - protein, 120 aa, Artificial Sequence
  Description of Artificial Sequences; note = synthetic construct
GFGTIRDTLNNKRKELEDSGTYNYPFTWNTPSAPPGYNIAVKPDQMQYTELSNAKMAYKQNKANIAQEQQYGSNEENIPADLENLQREIKVAQERLDMAIQAYNNQNNPGSSSREKKSKA

SEQ ID NO: 75 - protein, 120 aa, Artificial Sequence
  Description of Artificial Sequences; note = synthetic construct
PYLVDCFVSRPTEKTIFIIFMLVVGLISLVLNLLELVHLLCRCLSRGMRARQGQDAPPTQGTSSDPYTDQVFFYLPVGQGPSSPPCPTYNGLSSSEQNWANLTTEERLASSRPPLFLDPP

SEQ ID NO: 76 - protein, 120 aa, Artificial Sequence
  Description of Artificial Sequences; note = synthetic construct
CGSKEHGNRKMRGRLLLTYMASIFFKSVFEVAFLLIQWYLYGFTLSAVYICEQSPCPHRVDCFLSRPTEKTIFILFMLVVSMVSFVLNVIELFYVLFKAIKNHLGNEKEEVYCNPVELQK

SEQ ID NO: 77 - protein, 239 aa, Artificial Sequence
  Description of Artificial Sequences; note = synthetic construct
MVSKGEELFTGVVPILVELDGDVNGHKFSVSGEGEGDATYGKLTLKFICTTGKLPVPWPTLVTTLTYGVQCFSRYPDHMKQHDFFKSAMPEGYVQERTIFFKDDGNYKTRAEVKFEGDTLVNRIELKGIDFKEDGNILGHKLEYNYNSHNVYIMADKQKNGIKVNFKIRHNIEDGSVQLADHYQQNTPIGDGPVLLPDNHYLSTQSALSKDPNEKRDHMVLLEFVTAAGITLGMDELYK

SEQ ID NO: 78 - DNA, 60 bp, Artificial Sequence
  Description of Artificial Sequences; note = synthetic construct
ccctcctcccgggcctcctcccgggcctcctcccggccccggcccgacgacctggagatc

SEQ ID NO: 79 - DNA, 27 bp, Artificial Sequence
  Description of Artificial Sequences; note = synthetic construct
cggccccggcccgacgacctggagatc

SEQ ID NO: 80 - DNA, 27 bp, Artificial Sequence
  Description of Artificial Sequences; note = synthetic construct
cggccccggcccgacgacctggaggtg

SEQ ID NO: 81 - DNA, 27 bp, Artificial Sequence
  Description of Artificial Sequences; note = synthetic construct
cggccccggcccgacgacgtgcccgtg

SEQ ID NO: 82 - DNA, 27 bp, Artificial Sequence
  Description of Artificial Sequences; note = synthetic construct
aaggcccggtccgacgacctgtccgtg

SEQ ID NO: 83 - DNA, 48 bp, Artificial Sequence
  Description of Artificial Sequences; note = synthetic construct
cggcagcccaagatctggttccccaaccggcggaagccctggaagaag

SEQ ID NO: 84 - DNA, 108 bp, Artificial Sequence
  Description of Artificial Sequences; note = synthetic construct
cggcagcccaagatctggttccccaaccggcggaagccctggaagaagccctcctcccgggcctcctcccgggcctcctcccggccccggcccgacgacctggagatc

SEQ ID NO: 85 - DNA, 75 bp, Artificial Sequence
  Description of Artificial Sequences; note = synthetic construct
cggcagcccaagatctggttccccaaccggcggaagccctggaagaagcggccccggcccgacgacctggagatc

SEQ ID NO: 86 - DNA, 75 bp, Artificial Sequence
  Description of Artificial Sequences; note = synthetic construct
cggcagcccaagatctggttccccaaccggcggaagccctggaagaagcggccccggcccgacgacctggaggtg

SEQ ID NO: 87 - DNA, 75 bp, Artificial Sequence
  Description of Artificial Sequences; note = synthetic construct
cggcagcccaagatctggttccccaaccggcggaagccctggaagaagcggccccggcccgacgacgtgcccgtg

SEQ ID NO: 88 - DNA, 75 bp, Artificial Sequence
  Description of Artificial Sequences; note = synthetic construct
cggcagcccaagatctggttccccaaccggcggaagccctggaagaagaaggcccggtccgacgacctgtccgtg

SEQ ID NO: 89 - protein, 20 aa, Artificial Sequence
  Description of Artificial Sequences; note = synthetic construct
PCSRASSRMSSRARPDDLDV

SEQ ID NO: 90 - protein, 19 aa, Artificial Sequence
  Description of Artificial Sequences; note = synthetic construct
PRVSVPNFGRTQSSDSAYV

SEQ ID NO: 91 - protein, 26 aa, Artificial Sequence
  Description of Artificial Sequences; note = synthetic construct
  misc_feature (1)..(1): Xaa is biotinylated
  misc_feature (1)..(1): Xaa is L-2-aminohexanoic acid
XRQPKIWFPNRRKPWKKRPRPDDLEI